European Patent Application EP 4 212 624 A1, published July 19, 2023. Title: FUNCTIONAL FRAGMENT FOR REPROGRAMMING, COMPOSITION, AND APPLICATION THEREOF. Applicant: NEURAGEN BIOTHERAPEUTICS (SUZHOU) CO., LTD. Application EP21866017.3. The sequence listing filed with the application follows.

SEQUENCE LISTING (46 sequences)

SEQ ID NO: 1 - protein, 356 aa, Artificial Sequence
  Artificial Sequence
MTKSYSESGLMGEPQPQGPPSWTDECLSSQDEEHEADKKEDDLETMNAEEDSLRNGGEEEDEDEDLEEEEEEEEEDDDQKPKRRGPKKKKMTKARLERFKLRRMKANARERNRMHGLNAALDNLRKVVPCYSKTQKLSKIETLRLAKNYIWALSEILRSGKSPDLVSFVQTLCKGLSQPTTNLVAGCLQLNPRTFLPEQNQDMPPHLPTASASFPVHPYSYQSPGLPSPPYGTMDSSHVFHVKPPPHAYSAALEPFFESPLTDCTSPSFDGPLSPPLSINGNFSFKHEPSAEFEKNYAFTMHYPAATLAGAQSHGSIFSGTAAPRCEIPIDNIMSFDSHSHHERVMSAQLNAIFHD

SEQ ID NO: 2 - protein, 357 aa, Artificial Sequence
  Artificial Sequence
MTKSYSESGLMGEPQPQGPPSWTDECLSSQDEEHEADKKEDELEAMNAEEDSLRNGGEEEEEDEDLEEEEEEEEEEEDQKPKRRGPKKKKMTKARLERFKLRRMKANARERNRMHGLNAALDNLRKVVPCYSKTQKLSKIETLRLAKNYIWALSEILRSGKSPDLVSFVQTLCKGLSQPTTNLVAGCLQLNPRTFLPEQNPDMPPHLPTASASFPVHPYSYQSPGLPSPPYGTMDSSHVFHVKPPPHAYSAALEPFFESPLTDCTSPSFDGPLSPPLSINGNFSFKHEPSAEFEKNYAFTMHYPAATLAGPQSHGSIFSSGAAAPRCEIPIDNIMSFDSHSHHERVMSAQLNAIFHD

SEQ ID NO: 3 - DNA, 1071 bp, Artificial Sequence
  Artificial Sequence
atgaccaaatcgtacagcgagagtgggctgatgggcgagcctcagccccaaggtcctccaagctggacagacgagtgtctcagttctcaggacgaggagcacgaggcagacaagaaggaggacgacctcgaaaccatgaacgcagaggaggactcactgaggaacgggggagaggaggaggacgaagatgaggacctggaagaggaggaagaagaggaagaggaggatgacgatcaaaagcccaagagacgcggccccaaaaagaagaagatgactaaggctcgcctggagcgttttaaattgagacgcatgaaggctaacgcccgggagcggaaccgcatgcacggactgaacgcggcgctagacaacctgcgcaaggtggtgccttgctattctaagacgcagaagctgtccaaaatcgagactctgcgcttggccaagaactacatctgggctctgtcggagatcctgcgctcaggcaaaagcccagacctggtctccttcgttcagacgctttgcaagggcttatcccaacccaccaccaacctggttgcgggctgcctgcaactcaatcctcggacttttctgcctgagcagaaccaggacatgcccccccacctgccgacggccagcgcttccttccctgtacacccctactcctaccagtcgcctgggctgcccagtccgccttacggtaccatggacagctcccatgtcttccacgttaagcctccgccgcacgcctacagcgcagcgctggagcccttctttgaaagccctctgactgattgcaccagcccttcctttgatggacccctcagcccgccgctcagcatcaatggcaacttctctttcaaacacgaaccgtccgccgagtttgagaaaaattatgcctttaccatgcactatcctgcagcgacactggcaggggcccaaagccacggatcaatcttctcaggcaccgctgcccctcgctgcgagatccccatagacaatattatgtccttcgatagccattcacatcatgagcgagtcatgagtgcccagctcaatgccatatttcatgattag

SEQ ID NO: 4 - DNA, 1074 bp, Artificial Sequence
  Artificial Sequence
atgaccaaatcatacagcgagagcgggctgatgggcgagcctcagccccaaggtcccccaagctggacagatgagtgtctcagttctcaggacgaggaacacgaggcagacaagaaagaggacgagcttgaagccatgaatgcagaggaggactctctgagaaacgggggagaggaggaggaggaagatgaggatctagaggaagaggaggaagaagaagaggaggaggaggatcaaaagcccaagagacggggtcccaaaaagaaaaagatgaccaaggcgcgcctagaacgttttaaattaaggcgcatgaaggccaacgcccgcgagcggaaccgcatgcacgggctgaacgcggcgctggacaacctgcgcaaggtggtaccttgctactccaagacccagaaactgtctaaaatagagacactgcgcttggccaagaactacatctgggctctgtcagagatcctgcgctcaggcaaaagccctgatctggtctccttcgtacagacgctctgcaaaggtttgtcccagcccactaccaatttggtcgccggctgcctgcagctcaaccctcggactttcttgcctgagcagaacccggacatgcccccgcatctgccaaccgccagcgcttccttcccggtgcatccctactcctaccagtcccctggactgcccagcccgccctacggcaccatggacagctcccacgtcttccacgtcaagccgccgccacacgcctacagcgcagctctggagcccttctttgaaagccccctaactgactgcaccagcccttcctttgacggacccctcagcccgccgctcagcatcaatggcaacttctctttcaaacacgaaccatccgccgagtttgaaaaaaattatgcctttaccatgcactaccctgcagcgacgctggcagggccccaaagccacggatcaatcttctcttccggtgccgctgcccctcgctgcgagatccccatagacaacattatgtctttcgatagccattcgcatcatgagcgagtcatgagtgcccagcttaatgccatctttcacgattag

SEQ ID NO: 5 - protein, 443 aa, Artificial Sequence
  Artificial Sequence
MATAASNHYSLLTSSASIVHAEPPGGMQQGAGGYREAQSLVQGDYGALQSNGHPLSHAHQWITALSHGGGGGGGGGGGGGGGGGGGGGDGSPWSTSPLGQPDIKPSVVVQQGGRGDELHGPGALQQQHQQQQQQQQQQQQQQQQQQQQQRPPHLVHHAANHHPGPGAWRSAAAAAHLPPSMGASNGGLLYSQPSFTVNGMLGAGGQPAGLHHHGLRDAHDEPHHADHHPHPHSHPHQQPPPPPPPQGPPGHPGAHHDPHSDEDTPTSDDLEQFAKQFKQRRIKLGFTQADVGLALGTLYGNVFSQTTICRFEALQLSFKNMCKLKPLLNKWLEEADSSSGSPTSIDKIAAQGRKRKKRTSIEVSVKGALESHFLKCPKPSAQEITSLADSLQLEKEVVRVWFCNRRQKEKRMTPPGGTLPGAEDVYGGSRDTPPHHGVQTPVQ

SEQ ID NO: 6 - protein, 445 aa, Artificial Sequence
  Artificial Sequence
MATAASNHYSLLTSSASIVHAEPPGGMQQGAGGYREAQSLVQGDYGALQSNGHPLSHAHQWITALSHGGGGGGGGGGGGGGGGGGGGGDGSPWSTSPLGQPDIKPSVVVQQGGRGDELHGPGALQQQHQQQQQQQQQQQQQQQQQQQQQQQRPPHLVHHAANHHPGPGAWRSAAAAAHLPPSMGASNGGLLYSQPSFTVNGMLGAGGQPAGLHHHGLRDAHDEPHHADHHPHPHSHPHQQPPPPPPPQGPPGHPGAHHDPHSDEDTPTSDDLEQFAKQFKQRRIKLGFTQADVGLALGTLYGNVFSQTTICRFEALQLSFKNMCKLKPLLNKWLEEADSSSGSPTSIDKIAAQGRKRKKRTSIEVSVKGALESHFLKCPKPSAQEITSLADSLQLEKEVVRVWFCNRRQKEKRMTPPGGTLPGAEDVYGGSRDTPPHHGVQTPVQ

SEQ ID NO: 7 - DNA, 1332 bp, Artificial Sequence
  Artificial Sequence
atggcgaccgcagcgtctaaccactacagcctgctcacctccagcgcctccatcgtgcacgccgagccgcccggcggcatgcagcagggcgcggggggctaccgcgaagcgcagagcctggtgcagggcgactacggcgctctgcagagcaacggacacccgctcagccacgctcaccagtggatcaccgcgctgtcccacggcggcggcggcgggggcggtggcggcggcggggggggcgggggcggcggcgggggcggcggcgacggctccccgtggtccaccagccccctgggccagccggacatcaagccctcggtggtggtgcagcagggcggccgcggagacgagctgcacgggccaggcgccctgcagcagcagcatcagcagcagcaacagcaacagcagcagcaacagcagcaacagcagcagcagcagcagcaacagcggccgccgcatctggtgcaccacgccgctaaccaccacccgggacccggggcatggcggagcgcggcggctgcagcgcacctcccaccctccatgggagcgtccaacggcggcttgctctactcgcagcccagcttcacggtgaacggcatgctgggcgccggcgggcagccggccggtctgcaccaccacggcctgcgggacgcgcacgacgagccacaccatgccgaccaccacccgcacccgcactcgcacccacaccagcagccgccgcccccgccgcccccgcagggtccgcctggccacccaggcgcgcaccacgacccgcactcggacgaggacacgccgacctcggacgacctggagcagttcgccaagcagttcaagcagcggcggatcaaactgggatttacccaagcggacgtggggctggctctgggcaccctgtatggcaacgtgttctcgcagaccaccatctgcaggtttgaggccctgcagctgagcttcaagaacatgtgcaagctgaagcctttgttgaacaagtggttggaggaggcggactcgtcctcgggcagccccacgagcatagacaagatcgcagcgcaagggcgcaagcggaaaaagcggacctccatcgaggtgagcgtcaagggggctctggagagccatttcctcaaatgccccaagccctcggcccaggagatcacctccctcgcggacagcttacagctggagaaggaggtggtgagagtttggttttgtaacaggagacagaaagagaaaaggatgacccctcccggagggactctgccgggcgccgaggatgtgtacggggggagtagggacactccaccacaccacggggtgcagacgcccgtccagtga

SEQ ID NO: 8 - DNA, 1338 bp, Artificial Sequence
  Artificial Sequence
atggcgaccgcagcgtctaaccactacagcctgctcacctccagcgcctccatcgtacatgccgagccgcctggcggcatgcagcagggcgcagggggctaccgcgaggcgcagagcctggtgcagggcgactacggcgcgctgcagagcaacgggcacccgctcagccacgctcaccagtggatcaccgcgctgtcccacggcggcggcggcgggggcggcggcggcggtggaggaggcgggggaggcggcgggggaggcggcgacggctccccgtggtccaccagccccctaggccagccggacatcaagccctcggtggtggtacagcagggtggccgaggcgacgagctgcacgggccaggagcgctgcagcaacagcatcaacagcaacagcaacagcagcagcagcagcagcagcagcagcagcagcaacagcagcagcaacaacagcgaccgccacatctggtgcaccacgctgccaaccaccatcccgggcccggggcatggcggagtgcggcggctgcagctcacctccctccctccatgggagcttccaacggcggtttgctctattcgcagccgagcttcacggtgaacggcatgctgggcgcaggagggcagccggctgggctgcaccaccacggcctgagggacgcccacgatgagccacaccatgcagaccaccacccgcatccgcactctcacccacaccagcaaccgcccccgccacctcccccacaaggcccaccgggccacccaggcgcgcaccacgacccgcactcggacgaggacacgccgacctcagacgacctggagcagttcgccaagcaattcaagcagaggcggatcaaactcggatttactcaagcagacgtggggctggcgcttggcaccctgtacggcaacgtgttctcgcagaccaccatctgcaggtttgaggccctgcagctgagcttcaagaacatgtgcaagctgaagcctttgttgaacaagtggttggaagaggcagactcatcctcgggcagccccaccagcatagacaagatcgcagcgcaagggcgcaaacggaaaaagcggacctccatcgaggtgagcgtcaagggggctctggagagccatttcctcaaatgccctaagccctcggcccaggagatcacctccctcgcggacagcttacagctggagaaggaggtggtgagagtttggttttgtaacaggagacagaaagagaaaaggatgacccctcccggagggactctgccgggcgccgaggatgtgtatgggggtagtagggacacgccaccacaccacggggtgcagacgcccgtccagtga

SEQ ID NO: 9 - protein, 236 aa, Artificial Sequence
  Artificial Sequence
MESSAKMESGGAGQQPQPQPQQPFLPPAACFFATAAAAAAAAAAAAAQSAQQQQQQQQQQQQAPQLRPAADGQPSGGGHKSAPKQVKRQRSSSPELMRCKRRLNFSGFGYSLPQQQPAAVARRNERERNRVKLVNLGFATLREHVPNGAANKKMSKVETLRSAVEYIRALQQLLDEHDAVSAAFQAGVLSPTISPNYSNDLNSMAGSPVSSYSSDEGSYDPLSPEEQELLDFTNWF

SEQ ID NO: 10 - protein, 231 aa, Artificial Sequence
  Artificial Sequence
MESSGKMESGAGQQPQPPQPFLPPAACFFATAAAAAAAAAAAAQSAQQQQPQAPPQQAPQLSPVADSQPSGGGHKSAAKQVKRQRSSSPELMRCKRRLNFSGFGYSLPQQQPAAVARRNERERNRVKLVNLGFATLREHVPNGAANKKMSKVETLRSAVEYIRALQQLLDEHDAVSAAFQAGVLSPTISPNYSNDLNSMAGSPVSSYSSDEGSYDPLSPEEQELLDFTNWF

SEQ ID NO: 11 - DNA, 711 bp, Artificial Sequence
  Artificial Sequence
atggaaagctctgccaagatggagagcggcggcgccggccagcagccccagccgcagccccagcagcccttcctgccgcccgcagcctgtttctttgccacggccgcagccgcggcggccgcagccgccgcagcggcagcgcagagcgcgcagcagcagcagcagcagcagcagcagcagcagcaggcgccgcagctgagaccggcggccgacggccagccctcagggggcggtcacaagtcagcgcccaagcaagtcaagcgacagcgctcgtcttcgcccgaactgatgcgctgcaaacgccggctcaacttcagcggctttggctacagcctgccgcagcagcagccggccgccgtggcgcgccgcaacgagcgcgagcgcaaccgcgtcaagttggtcaacctgggctttgccacccttcgggagcacgtccccaacggcgcggccaacaagaagatgagtaaggtggagacactgcgctcggcggtcgagtacatccgcgcgctgcagcagctgctggacgagcatgacgcggtgagcgccgccttccaggcaggcgtcctgtcgcccaccatctcccccaactactccaacgacttgaactccatggccggctcgccggtctcatcctactcgtcggacgagggctcttacgacccgctcagccccgaggagcaggagcttctcgacttcaccaactggttctga

SEQ ID NO: 12 - DNA, 696 bp, Artificial Sequence
  Artificial Sequence
atggagagctctggcaagatggagagtggagccggccagcagccgcagcccccgcagcccttcctgcctcccgcagcctgcttctttgcgaccgcggcggcggcggcagcggcggcggccgcggcagctcagagcgcgcagcagcaacagccgcaggcgccgccgcagcaggcgccgcagctgagcccggtggccgacagccagccctcagggggcggtcacaagtcagcggccaagcaggtcaagcgccagcgctcgtcctctccggaactgatgcgctgcaaacgccggctcaacttcagcggcttcggctacagcctgccacagcagcagccggccgccgtggcgcgccgcaacgagcgcgagcgcaaccgggtcaagttggtcaacctgggttttgccaccctccgggagcatgtccccaacggcgcggccaacaagaagatgagcaaggtggagacgctgcgctcggcggtcgagtacatccgcgcgctgcagcagctgctggacgagcacgacgcggtgagcgctgcctttcaggcgggcgtcctgtcgcccaccatctcccccaactactccaacgacttgaactctatggcgggttctccggtctcgtcctactcctccgacgagggatcctacgaccctcttagcccagaggaacaagagctgctggactttaccaactggttctga

SEQ ID NO: 13 - protein, 272 aa, Artificial Sequence
  Artificial Sequence
MFVKSETLELKEEEDVLVLLGSASPALAALTPLSSSADEEEEEEPGASGGARRQRGAEAGQGARGGVAAGAEGCRPARLLGLVHDCKRRPSRARAVSRGAKTAETVQRIKKTRRLKANNRERNRMHNLNAALDALREVLPTFPEDAKLTKIETLRFAHNYIWALTETLRLADHCGGGGGGLPGALFSEAVLLSPGGASAALSSSGDSPSPASTWSCTNSPAPSSSVSSNSTSPYSCTLSPASPAGSDMDYWQPPPPDKHRYAPHLPIARDCI

SEQ ID NO: 14 - protein, 263 aa, Artificial Sequence
  Artificial Sequence
MFVKSETLELKEEEEVLMLLGSASPASATLTPMSSSADEEEDEELRRPGSARGQRGAEAGQGVQGSPASGAGGCRPGRLLGLMHECKRRPSRSRAVSRGAKTAETVQRIKKTRRLKANNRERNRMHNLNAALDALREVLPTFPEDAKLTKIETLRFAHNYIWALTETLRLADHCAGAGGLQGALFTEAVLLSPGAALGASGDSPSPPSSWSCTNSPASSSNSTSPYSCTLSPASPGSDVDYWQPPPPEKHRYAPHLPLARDCI

SEQ ID NO: 15 - DNA, 819 bp, Artificial Sequence
  Artificial Sequence
atgttcgtcaaatccgagaccttggagttgaaggaggaagaggacgtgttagtgctgctcggatcggcctcccccgccttggcggccctgaccccgctgtcatccagcgccgacgaagaagaggaggaggagccgggcgcgtcaggcggggcgcgtcggcagcgcggggctgaggccgggcagggggcgcggggcggcgtggctgcgggtgcggagggctgccggcccgcacggctgctgggtctggtacacgattgcaaacggcgcccttcccgggcgcgggccgtctcccgaggcgccaagacggccgagacggtgcagcgcatcaagaagacccgtagactgaaggccaacaaccgcgagcgaaaccgcatgcacaacctcaacgcggcactggacgcgctgcgcgaggtgctccccacgttccccgaggacgccaagctcaccaagatcgagaccctgcgcttcgcccacaactacatctgggcactcaccgagaccctgcgcctggcggatcactgcgggggcggcggcgggggcctgccgggggcgctcttctccgaggcagtgttgctgagcccgggaggagccagcgccgccctgagcagcagcggagacagcccctcgcccgcctccacgtggagttgcaccaacagccccgcgccgtcctcctccgtgtcctccaattccacctccccctacagctgcactttatcgcccgccagcccggccgggtcagacatggactattggcagcccccacctcccgacaagcaccgctatgcacctcacctccccatagccagggattgtatctag

SEQ ID NO: 16 - DNA, 792 bp, Artificial Sequence
  Artificial Sequence
atgttcgtcaaatctgagactctggagttgaaggaggaagaggaggtactgatgctgctgggctcggcttccccggcctcggcgaccctgaccccgatgtcctccagcgcggacgaggaggaggacgaggagctgcgccggccgggctccgcgcgtgggcagcgtggagcggaagccgggcagggggtgcagggcagtccggcgtcgggtgccgggggttgccggccagggcggctgctgggcctgatgcacgagtgcaagcgtcgcccgtcgcgctcacgggccgtctcccgaggtgccaagacggcggagacggtgcagcgcatcaagaagacccgcaggctcaaggccaacaaccgcgagcgcaaccgcatgcacaacctaaacgccgcgctggacgcgctgcgcgaggtgctgcccaccttccccgaggatgccaagctcacgaagatcgagacgctgcgcttcgcccacaattacatctgggcgctcaccgagactctgcgcctggcggaccactgcgccggcgccggtggcctccagggggcgctcttcacggaggcggtgctcctgagcccgggagctgcgctcggcgccagcggggacagcccttctccaccttcctcctggagctgcaccaacagcccggcgtcatcctccaactccacgtccccatacagctgcactttatcgcccgctagccccgggtcagacgtggactactggcagcccccacctccggagaagcatcgttatgcgcctcacctgcccctcgccagggactgtatctag

SEQ ID NO: 17 - protein, 264 aa, Artificial Sequence
  Artificial Sequence
MPRSFLVDSLVLREAGEKKAPEGSPPPLFPYAVPPPHALHGLSPGACHARKAGLLCVCPLCVTASQLHGPPGPPALPLLKASFPPFGSQYCHAPLGRQHSAVSPGVAHGPAAAAAAAALYQTSYPLPDPRQFHCISVDSSSNQLPSSKRMRTAFTSTQLLELEREFASNMYLSRLRRIEIATYLNLSEKQVKIWFQNRRVKHKKEGKGSNHRGGGGGGAGGGGSAPQGCKCASLSSAKCSEDDDELPMSPSSSGKDDRDLTVTP

SEQ ID NO: 18 - protein, 261 aa, Artificial Sequence
  Artificial Sequence
MPRSFLVDSLVLREASDKKAPEGSPPPLFPYAVPPPHALHGLSPGACHARKAGLLCVCPLCVTASQLHGPPGPPALPLLKASFPPFGSQYCHAPLGRQHSVSPGVAHGPAAAAAAAALYQTSYPLPDPRQFHCISVDSSSNQLPSSKRMRTAFTSTQLLELEREFASNMYLSRLRRIEIATYLNLSEKQVKIWFQNRRVKHKKEGKGSNHRGGAGAGAGGGAPQGCKCSSLSSAKCSEDDDELPMSPSSSGKDDRDLTVTP

SEQ ID NO: 19 - DNA, 795 bp, Artificial Sequence
  Artificial Sequence
atgccgcgctccttcctggtggactcgctagtgctgcgcgaggcgggcgagaagaaggcgcccgagggcagcccgccgccgctcttcccctacgctgtgcccccgccgcacgcgctgcacggtctctcgcctggcgcctgccacgcgcgcaaggctgggctgctgtgcgtgtgcccgctctgcgtcaccgcctcgcagctgcatgggccccccgggccgcccgcgctgcctctactcaaggcttccttcccacccttcggctcgcagtactgccacgcgcccctgggccgccagcactctgctgtgtcgcccggggtcgctcacggcccggccgccgctgctgctgccgccgcgctctaccagacctcctacccgctgcctgaccccaggcagttccactgcatctctgtggacagcagctctaaccagctgcccagcagcaagaggatgcgcacggctttcaccagcacgcagctgctagagctggagcgcgagttcgcttctaatatgtacctgtcccgcctacgtcgcatcgagatcgcgacctacctgaatctgtccgagaagcaggtgaagatctggtttcagaaccgccgagtgaagcacaagaaggagggcaagggcagcaaccatcgtggcggcggcggcgggggtgccggtggtggcgggagcgcaccgcaaggctgcaagtgcgcatcgctctcctcagccaagtgctccgaggatgacgacgaattgcccatgtctccgtcctcctcagggaaggacgaccgggatcttacggtcactccctag

SEQ ID NO: 20 - DNA, 786 bp, Artificial Sequence
  Artificial Sequence
atgccgcgctccttcctggtggattcccttgtgctgcgggaagccagcgacaagaaggctccggagggcagcccgccaccgctcttcccctacgcggtcccgccgccgcacgcgctccacggcctctcgccgggcgcctgccacgcgcgcaaggccggcttgctgtgcgtgtgtcccctctgtgtcaccgcttcgcagctgcacgggccccccgggccgccggcactgccgctactcaaggcgtccttccctcccttcggatcgcagtactgccacgcacccctgggccgccagcactccgtgtcccctggagtcgcccacggcccggctgcggccgcagcagctgctgcactctaccagacctcctacccgctgccggatcccagacagtttcactgcatctctgtggacagcagctcgaaccagctgcccagcagcaagaggatgcggacggcgttcaccagcacacagctcctggagctggagcgagagttcgcctccaacatgtacctctcccgcctgcggcgcatcgagatcgcgacctatctgaacctgtccgagaagcaggtgaagatctggtttcagaaccgccgggtgaagcacaagaaagaaggcaaaggcagtaaccaccgcggcggagctggggcgggggccggcgggggcgcaccgcaaggctgcaagtgctcttcgctctcctcagccaaatgctcagaggacgacgacgaattgcccatgtctccatcttcctccgggaaggatgacagagatctcacagtcactccgtag

SEQ ID NO: 21 - protein, 682 aa, Artificial Sequence
  Artificial Sequence
MQLEHCLSPSIMLSKKFLNVSSSYPHSGGSELVLHDHPIISTTDNLERSSPLKKITRGMTNQSDTDNFPDSKDSPGDVQRSKLSPVLDGVSELRHSFDGSAADRYLLSQSSQPQSAATAPSAMFPYPGQHGPAHPAFSIGSPSRYMAHHPVITNGAYNSLLSNSSPQGYPTAGYPYPQQYGHSYQGAPFYQFSSTQPGLVPGKAQVYLCNRPLWLKFHRHQTEMIITKQGRRMFPFLSFNISGLDPTAHYNIFVDVILADPNHWRFQGGKWVPCGKADTNVQGNRVYMHPDSPNTGAHWMRQEISFGKLKLTNNKGASNNNGQMVVLQSLHKYQPRLHVVEVNEDGTEDTSQPGRVQTFTFPETQFIAVTAYQNTDITQLKIDHNPFAKGFRDNYDTIYTGCDMDRLTPSPNDSPRSQIVPGARYAMAGSFLQDQFVSNYAKARFHPGAGAGPGPGTDRSVPHTNGLLSPQQAEDPGAPSPQRWFVTPANNRLDFAASAYDTATDFAGNAATLLSYAAAGVKALPLQAAGCTGRPLGYYADPSGWGARSPPQYCGTKSGSVLPCWPNSAAAAARMAGANPYLGEEAEGLAAERSPLPPGAAEDAKPKDLSDSSWIETPSSIKSIDSSDSGIYEQAKRRRISPADTPVSESSSPLKSEVLAQRDCEKNCAKDISGYYGFYSHS

SEQ ID NO: 22 - protein, 681 aa, Artificial Sequence
  Artificial Sequence
MQLEHCLSPSIMLSKKFLNVSSSYPHSGGSELVLHDHPIISTTDNLERSSPLKKITRGMTNQSDTDNFPDSKDSPGDVQRSKLSPVLDGVSELRHSFDGSAADRYLLSQSSQPQSAATAPSAMFPYPSQHGPAHPAFSIGSPSRYMAHHPVITNGAYNSLLSNSSPQGYPTAGYPYPQQYGHSYQGAPFYQFSSTQPGLVPGKAQVYLCNRPLWLKFHRHQTEMIITKQGRRMFPFLSFNISGLDPTAHYNIFVDVILADPNHWRFQGGKWVPCGKADTNVQGNRVYMHPDSPNTGAHWMRQEISFGKLKLTNNKGASNNNGQMVVLQSLHKYQPRLHVVEVNEDGTEDTSQPGRVQTFTFPETQFIAVTAYQNTDITQLKIDHNPFAKGFRDNYDTIYTGCDMDRLTPSPNDSPRSQIVPGARYAMAGSFLQDQFVSNYAKARFHPGAGAGPGPGTDRSVPHTNGLLSPQQAEDPGAPSPQRWFVTPANNRLDFAASAYDTATDFAGNAATLLSYAAAGVKALPLQAAGCTGRPLGYYADPSGWGARSPPQYCGAKSGSVLPCWPNSAAAAARMAGANPYLGEEAEGLAAERSPLAPAAEDAKPKDLSDSSWIETPSSIKSIDSSDSGIYEQAKRRRISPADTPVSESSSPLKSEVLAQRDCEKNCAKDIGGYYGFYSHS

SEQ ID NO: 23 - DNA, 2049 bp, Artificial Sequence
  Artificial Sequence
atgcagctggagcactgcctttctccttctatcatgctctccaagaaatttctcaatgtgagcagcagctacccacattcaggcggatccgagcttgtcttgcacgatcatcccattatctcgaccactgacaacctggagagaagttcacctttgaaaaaaattaccagggggatgacgaatcagtcagatacagacaattttcctgactccaaggactcaccaggggacgtccagagaagtaaactctctcctgtcttggacggggtctctgagcttcgtcacagtttcgatggctctgctgcagatcgctacctcctctctcagtccagccagccacagtctgcggccactgctcccagtgccatgttcccgtaccccggccagcacggaccggcgcaccccgccttctccatcggcagccctagccgctacatggcccaccacccggtcatcaccaacggagcctacaacagcctcctgtccaactcctcgccgcagggataccccacggccggctacccctacccacagcagtacggccactcctaccaaggagctccgttctaccagttctcctccacccagccggggctggtgcccggcaaagcacaggtgtacctgtgcaacaggcccctttggctgaaatttcaccggcaccaaacggagatgatcatcaccaaacagggaaggcgcatgtttccttttttaagttttaacatttctggtctcgatcccacggctcattacaatatttttgtggatgtgattttggcggatcccaatcactggaggtttcaaggaggcaaatgggttccttgcggcaaagcggacaccaatgtgcaaggaaatcgggtctatatgcatccggattcccccaacactggggctcactggatgcgccaagaaatctcttttggaaaattaaaacttacgaacaacaaaggagcttcaaataacaatgggcagatggtggttttacagtccttgcacaagtaccagccccgcctgcatgtggtggaagtgaacgaggacggcacggaggacactagccagcccggccgcgtgcagacgttcactttccctgagactcagttcatcgccgtcaccgcctaccagaacacggatattacacaactgaaaatagatcacaacccttttgcaaaaggatttcgggataattatgacacgatctacaccggctgtgacatggaccgcctgaccccctcgcccaacgactcgccgcgctcgcagatcgtgcccggggcccgctacgccatggccggctctttcctgcaggaccagttcgtgagcaactacgccaaggcccgcttccacccgggcgcgggcgcgggccccgggccgggtacggaccgcagcgtgccgcacaccaacgggctgctgtcgccgcagcaggccgaggacccgggcgcgccctcgccgcaacgctggtttgtgacgccggccaacaaccggctggacttcgcggcctcggcctatgacacggccacggacttcgcgggcaacgcggccacgctgctctcttacgcggcggcgggcgtgaaggcgctgccgctgcaggctgcaggctgcactggccgcccgctcggctactacgccgacccgtcgggctggggcgcccgcagtcccccgcagtactgcggcaccaagtcgggctcggtgctgccctgctggcccaacagcgccgcggccgccgcgcgcatggccggcgccaatccctacctgggcgaggaggccgagggcctggccgccgagcgctcgccgctgccgcccggcgccgccgaggacgccaagcccaaggacctgtccgattccagctggatcgagacgccctcctcgatcaagtccatcgactccagcgactcggggatttacgagcaggccaagcggaggcggatctcgccggccgacacgcccgtgtccgagagttcgtccccgctcaagagcgaggtgctggcccagcgggactgcgagaagaactgcgccaaggacattagcggctactatggcttctactcgcacagctag

SEQ ID NO: 24 - DNA, 2046 bp, Artificial Sequence
  Artificial Sequence
atgcagctggagcattgcctctctccttctatcatgctctccaagaaatttctcaatgtgagcagcagctacccacattcgggcggatctgagcttgtcttgcatgatcatcccattatctcgaccactgacaacctggagagaagttcacctttgaaaaaaattaccagggggatgacgaatcagtcagatacagacaattttcctgactccaaggactcaccaggggacgtccagagaagtaaactctctcctgtcttggacggggtctctgagcttcgtcacagtttcgatggctctgctgcagatcgttacctactctctcagtccagccagccacagtctgcggccaccgctcccagtgccatgttcccgtaccccagccagcacggaccggcgcatcccgccttctccatcggcagccccagtcgctacatggcccaccacccggtcattaccaacggagcttacaacagcctgctgtccaactcttcgccgcagggctaccccacggccggctacccctacccacagcagtacggccactcctaccaaggagcccctttctaccagttctcctccacccagcccgggttggtgcccggcaaggcgcaagtatacctgtgcaacaggccactttggctgaaatttcatcggcatcaaacggagatgatcatcactaaacagggaaggcgcatgtttccctttttgagttttaacatttctggtctcgatcccaccgctcattacaatatttttgtggatgtgattttggcggatcccaatcactggaggtttcaaggaggcaaatgggttccttgtggcaaagcggacaccaatgtgcaaggaaaccgggtctatatgcatccggattcccccaacactggggctcactggatgcggcaagaaatctcttttggaaaattaaaacttaccaacaacaagggagcatcaaacaacaatgggcagatggtggttttacagtccctgcacaagtaccagccccgtctgcacgtggtggaagtgaatgaggatggcacagaggacaccagccagccaggccgagtccagacgttcacttttccggagactcagttcatcgctgtcaccgcctaccagaacacggatattacacaactaaaaatagatcataacccctttgcaaaaggatttcgagataactatgacacgatctacacgggctgcgacatggaccgcttgaccccgtcgcccaacgactctccgcgctcgcagatcgtgcccggcgcccgctacgccatggccggctctttcctgcaagaccagttcgtgagcaactacgccaaggcccgcttccacccgggcgccggcgcgggtcccgggccgggcacggaccgcagcgtgccgcacaccaacgggctgctgtccccgcagcaggccgaggacccgggcgcgccgtcgccgcagcgctggttcgtcacgccggccaacaaccggctggacttcgcggcctcggcctacgacacggccacggacttcgccggcaacgcggccacgctgctgtcgtatgcggccgcgggcgtgaaggcgctgcccttgcaggccgcgggctgcacgggccgcccgctcggctactacgccgacccttcgggctggggcgcgcgcagccccccgcagtactgcggcgccaagtcgggctccgtgctcccctgctggcccaacagcgccgcggccgccgcgcgcatggccggcgccaacccctatctgggcgaggaggccgagggcctggcggccgagcgctcgccgctggcgcccgccgccgaggacgccaagcccaaggacctgtccgactccagctggatcgagacgccctcctccatcaaatccatcgactccagcgactcggggatttacgagcaggccaagcggaggcggatctcgccggctgacacgccggtgtctgagagctcgtccccgctcaagagcgaggtgctggcccagcgggactgcgagaagaactgcgccaaggacataggcggctactatggcttctactcgcacagctag

SEQ ID NO: 25 - protein, 328 aa, Artificial Sequence
  Artificial Sequence
MTGVFDSLVADMHSTQIAASSTYHQHQQPPSGGGAGPGGNSSSSSSLHKPQESPTLPVSTATDSSYYTNQQHPAGGGGGGGSPYAHMGSYQYQASGLNNVPYSAKSSYDLGYTAAYTSYAPYGTSSSPANNEPEKEDLEPEIRIVNGKPKKVRKPRTIYSSFQLAALQRRFQKTQYLALPERAELAASLGLTQTQVKIWFQNRRSKFKKMWKSGEIPSEQHPGASASPPCASPPVSAPASWDFGVPQRMAGGGGPGSGGSGAGSSGSSPSSAASAFLGNYPWYHQTSGSASHLQATAPLLHPTQTPQPHHHHHHHGGGGAPVSAGTIF

SEQ ID NO: 26 - protein, 332 aa, Artificial Sequence
  Artificial Sequence
MTGVFDSLVADMHSTQITASSTYHQHQQPPSGAGAGPGGNSNSSSSNSSLHKPQESPTLPVSTATDSSYYTNQQHPAGGGGGGASPYAHMGSYQYHASGLNNVSYSAKSSYDLGYTAAYTSYAPYGTSSSPVNNEPDKEDLEPEIRIVNGKPKKVRKPRTIYSSFQLAALQRRFQKTQYLALPERAELAASLGLTQTQVKIWFQNRRSKFKKMWKSGEIPTEQHPGASASPPCASPPVSAPASWDFGAPQRMAGGGPGSGGGGAGSSGSSPSSAASAFLGNYPWYHQASGSASHLQATAPLLHPSQTPQAHHHHHHHHHAGGGAPVSAGTIF

SEQ ID NO: 27 - DNA, 987 bp, Artificial Sequence
  Artificial Sequence
atgactggagtctttgacagtctagtggctgatatgcactcgacccagatcgccgcctccagcacgtaccaccagcaccagcagcccccgagcggcggcggcgccggcccgggtggcaacagcagcagcagcagcagcctccacaagccccaggagtcgcccacccttccggtgtccaccgccaccgacagcagctactacaccaaccagcagcacccggcgggcggcggcggcggcgggggctcgccctacgcgcacatgggttcctaccagtaccaagccagcggcctcaacaacgtcccttactccgccaagagcagctatgacctgggctacaccgccgcctacacctcctacgctccctatggaaccagttcgtccccagccaacaacgagcctgagaaggaggaccttgagcctgaaattcggatagtgaacgggaagccaaagaaagtccggaaaccccgcaccatctactccagtttccagctggcggctcttcagcggcgtttccaaaagactcaatacttggccttgccggagcgagccgagctggcggcctctctgggcctcacccagactcaggtcaaaatctggttccagaaccgccggtccaagttcaagaagatgtggaaaagtggtgagatcccctcggagcagcaccctggggccagcgcttctccaccttgtgcttcgccgccagtctcagcgccggcctcctgggactttggtgtgccgcagcggatggcgggcggcggtggtccgggcagtggcggcagcggcgccggcagctcgggctccagcccgagcagcgcggcctcggcttttctgggcaactacccctggtaccaccagacctcgggatccgcctcacacctgcaggccacggcgccgctgctgcaccccactcagaccccgcagccgcatcaccaccaccaccatcacggcggcgggggcgccccggtgagcgcggggacgattttctaa

SEQ ID NO: 28 - DNA, 999 bp, Artificial Sequence
  Artificial Sequence
atgactggagtctttgacagtctggtggctgatatgcactcgacccagatcaccgcctccagcacgtaccaccagcaccagcagcccccgagcggtgcgggcgccggccctggcggcaacagcaacagcagcagcagcaacagcagcctgcacaagccccaggagtcgccaaccctcccggtgtccacggctacggacagcagctactacaccaaccagcagcacccggcgggcggcggcggcgggggggcctcgccctacgcgcacatgggctcctaccagtaccacgccagcggcctcaacaatgtctcctactccgccaaaagcagctacgacctgggctacaccgccgcgtacacctcctacgcgccctacggcaccagttcgtctccggtcaacaacgagccggacaaggaagaccttgagcctgaaatccgaatagtgaacgggaagccaaagaaagtccggaaaccacgcaccatctactccagtttccagctggcggcccttcaacgacgcttccagaagacccagtatctggccctgccagagcgagccgagctggcggcgtccctgggcctcacccaaactcaggtcaaaatctggttccagaaccgccgatccaagttcaagaagatgtggaaaagcggcgagatacccaccgagcagcaccctggagccagcgcttctcctccttgtgcctccccgccggtctcggcgccagcatcctgggacttcggcgcgccgcagcggatggctggcggcggcccgggcagcggaggcggcggtgcgggcagctctggctccagcccgagcagcgccgcctcggcctttctgggaaactacccgtggtaccaccaggcttcgggctccgcttcacacctgcaggccacagcgccacttctgcatccttcgcagactccgcaggcgcaccatcaccaccatcaccaccaccacgcaggcgggggcgccccggtgagcgcggggacgattttctaa

SEQ ID NO: 29 - protein, 328 aa, Artificial Sequence
  Artificial Sequence
MDAVLLEHFPGGLDAFPSSYFDEDDFFTDQSSRDPLEDGDELLADEQAEVEFLSHQLHEYCYRDGACLLLQPAPPAAPLALAPPSSGGLGEPDDGGGGGYCCETGAPPGGFPYSPGSPPSCLAYPCAGAAVLSPGARLRGLSGAAAAAARRRRRVRSEAELQQLRQAANVRERRRMQSINDAFEGLRSHIPTLPYEKRLSKVDTLRLAIGYINFLSELVQADLPLRGGGAGGCGGPGGGGRLGGDSPGSQAQKVIICHRGTRSPSPSDPDYGLPPLAGHSLSWTDEKQLKEQNIIRTAKVWTPEDPRKLNSKSSFNNIENEPPFEFVS

SEQ ID NO: 30 - protein, 324 aa, Artificial Sequence
  Artificial Sequence
MDAVLLEHFPGGLDTFPSPYFDEEDFFTDQSSRDPLEDSDELLGDEQAEVEFLSHQLHEYCYRDGACLLLQPAPSAAPHALAPPPLGDPGEPEDNVSYCCDAGAPLAAFPYSPGSPPSCLAYPCAAVLSPGARLGGLNGAAAAAAARRRRRVRSEAELQQLRQAANVRERRRMQSINDAFEGLRSHIPTLPYEKRLSKVDTLRLAIGYINFLSELVQADLPLRGSGAGGCGGPGGSRHLGEDSPGNQAQKVIICHRGTRSPSPSDPDYGLPPLAGHSLSWTDEKQLKEQNIIRTAKVWTPEDPRKLNSKSFDNIENEPPFEFVS

SEQ ID NO: 31 - DNA, 987 bp, Artificial Sequence
  Artificial Sequence
atggacgcggtgttgctggagcacttccccgggggcctagacgcctttccttcttcgtacttcgacgaggacgacttcttcaccgaccagtcttcacgggaccccctggaggacggcgatgagctgctggcggacgagcaggccgaggtggagttccttagccaccagctccacgagtactgctaccgcgacggggcgtgcctgctgctgcagcccgcgcccccggccgccccgctagcgctcgccccgccgtcctcggggggcctcggtgagccagacgacggcggcggcggcggctactgctgcgagacgggggcgcccccaggcggcttcccctactcgcccggctcgccgccctcgtgcctggcctacccgtgcgccggggcggcagtactgtctcccggggcgcggctgcgcggcctgagcggagcggcggctgcggcggcgcggcgccggcggcgggtgcgctccgaggcggagctgcagcagctgcggcaggcggccaacgtgcgcgagcggcggcgcatgcagtccatcaacgacgccttcgaggggctgcgctcgcacatccccacgctgccctacgagaagcgcctctccaaggtggacacgctgcgcctggccatcggctacatcaacttcctcagcgagctcgtgcaggccgacctgcccttgcgcggcggtggcgcgggcggctgcggggggccgggcggcggcgggcgcctgggcggggacagcccgggcagccaggcccagaaggtcatcatctgccatcggggcacccggtccccctcccccagcgaccctgattatggcctccctcccctagcaggacactctctctcatggactgatgaaaaacaactcaaggaacaaaatattatccgaacagccaaagtctggaccccagaggaccccagaaaactcaacagcaaatcttccttcaacaacatagaaaacgaaccaccatttgagtttgtgtcctga

SEQ ID NO: 32 - DNA, 975 bp, Artificial Sequence
  Artificial Sequence
atggacgccgtactcctggagcacttccccgggggcctggacaccttcccatccccttactttgatgaggaagatttcttcaccgaccagtcctctcgggacccgctggaggacagcgacgagctgctgggggacgagcaagcagaagtagagttcctcagccaccagctacacgaatactgctaccgcgacggggcgtgcctgctgctgcaacccgcgccctcggccgccccgcacgcgctcgccccgccgcctttgggggatcctggcgagcccgaggacaacgtcagctattgctgcgatgcaggggctcctctcgctgccttcccctactcgcctggctcaccgccctcgtgcctcgcctacccgtgtgccgcggtgctgtcccccggtgcgcggctcggtggtttgaacggggctgcggcagcggcggcagcaaggcggcggcgacgcgtgcgctccgaggcggagctgcagcagctgcgacaagccgctaatgtgcgagagcggcgccgcatgcagtccatcaacgacgccttcgaggggctgcgttcgcacatccccacgctaccctacgaaaagcgcctctccaaagtagacacgctgcgcttggccataggctacattaacttcctcagcgagctggtgcaagccgacctgccgctgcgcgggagtggcgcaggtggttgcgggggcccaggtggcagccggcacctcggagaggacagtcccggtaaccaggcccagaaggttatcatctgccatcgaggcacccgttcaccctcccccagtgacccggattatggtctccctcctcttgcagggcactctctttcctggactgatgaaaaacagctcaaagaacaaaatatcatccgtacagctaaagtgtggaccccagaggaccccagaaaactcaacagtaaatctttcgacaacatagagaacgaaccaccctttgagtttgtgtcctga

SEQ ID NO: 33 - protein, 422 aa, Artificial Sequence [sequence omitted]

SEQ ID NO: 34 - protein, 436 aa, Artificial Sequence
  Artificial Sequence
MQNSHSGVNQLGGVFVNGRPLPDSTRQKIVELAHSGARPCDISRILQTHADAKVQVLDNENVSNGCVSKILGRYYETGSIRPRAIGGSKPRVATPEVVSKIAQYKRECPSIFAWEIRDRLLSEGVCTNDNIPSVSSINRVLRNLASEKQQMGADGMYDKLRMLNGQTGSWGTRPGWYPGTSVPGQPTQDGCQQQEGGGENTNSISSNGEDSDEAQMRLQLKRKLQRNRTSFTQEQIEALEKEFERTHYPDVFARERLAAKIDLPEARIQVWFSNRRAKWRREEKLRNQRRQASNTPSHIPISSSFSTSVYQPIPQPTTPVSSFTSGSMLGRTDTALTNTYSALPPMPSFTMANNLPMQPPVPSQTSSYSCMLPTSPSVNGRSYDTYTPPHMQTHMNSQPMGTSGTTSTGLISPGVSVPVQVPGSEPDMSQYWPRLQ

SEQ ID NO: 35 - DNA, 1269 bp, Artificial Sequence
  Artificial Sequence
atgcagaacagtcacagcggagtgaatcagctcggtggtgtctttgtcaacgggcggccactgccggactccacccggcagaagattgtagagctagctcacagcggggcccggccgtgcgacatttcccgaattctgcaggtgtccaacggatgtgtgagtaaaattctgggcaggtattacgagactggctccatcagacccagggcaatcggtggtagtaaaccgagagtagcgactccagaagttgtaagcaaaatagcccagtataagcgggagtgcccgtccatctttgcttgggaaatccgagacagattactgtccgagggggtctgtaccaacgataacataccaagcgtgtcatcaataaacagagttcttcgcaacctggctagcgaaaagcaacagatgggcgcagacggcatgtatgataaactaaggatgttgaacgggcagaccggaagctggggcacccgccctggttggtatccggggacttcggtgccagggcaacctacgcaagatggctgccagcaacaggaaggagggggagagaataccaactccatcagttccaacggagaagattcagatgaggctcaaatgcgacttcagctgaagcggaagctgcaaagaaatagaacatcctttacccaagagcaaattgaggccctggagaaagagtttgagagaacccattatccagatgtgtttgcccgagaaagactagcagccaaaatagatctacctgaagcaagaatacaggtatggttttctaatcgaagggccaaatggagaagagaagaaaaactgaggaatcagagaagacaggccagcaacacacctagtcatattcctatcagcagtagtttcagcaccagtgtctaccaaccaattccacaacccaccacaccggtttcctccttcacatctggctccatgttgggccgaacagacacagccctcacaaacacctacagcgctctgccgcctatgcccagcttcaccatggcaaataacctgcctatgcaacccccagtccccagccagacctcctcatactcctgcatgctgcccaccagcccttcggtgaatgggcggagttatgatacctacacccccccacatatgcagacacacatgaacagtcagccaatgggcacctcgggcaccacttcaacaggactcatttcccctggtgtgtcagttccagttcaagttcccggaagtgaacctgatatgtctcaatactggccaagattacagtaa

SEQ ID NO: 36 - DNA, 1311 bp, Artificial Sequence
  Artificial Sequence
atgcagaacagtcacagcggagtgaatcagcttggtggtgtctttgtcaacgggcggccactgccggactccacccggcagaagatcgtagagctagctcacagcggggcccggccgtgcgacatttcccgaattctgcagacccatgcagatgcaaaagtccaggtgctggacaatgaaaacgtatccaacggttgtgtgagtaaaattctgggcaggtattacgagactggctccatcagacccagggcaatcggagggagtaagccaagagtggcgactccagaagttgtaagcaaaatagcccagtataaacgggagtgcccttccatctttgcttgggaaatccgagacagattattatccgagggggtctgtaccaacgataacatacccagtgtgtcatcaataaacagagttcttcgcaacctggctagcgaaaagcaacagatgggcgcagacggcatgtatgataaactaaggatgttgaacgggcagaccggaagctggggcacacgccctggttggtatcccgggacttcagtaccagggcaacccacgcaagatggctgccagcaacaggaaggagggggagagaacaccaactccatcagttctaacggagaagactcggatgaagctcagatgcgacttcagctgaagcggaagctgcaaagaaatagaacatcttttacccaagagcagattgaggctctggagaaagagtttgagaggacccattatccagatgtgtttgcccgggaaagactagcagccaaaatagatctacctgaagcaagaatacaggtatggttttctaatcgaagggccaaatggagaagagaagagaaactgaggaaccagagaagacaggccagcaacactcctagtcacattcctatcagcagcagcttcagtaccagtgtctaccagccaatcccacagcccaccacacctgtctcctccttcacatcaggttccatgttgggccgaacagacaccgccctcaccaacacgtacagtgctttgccacccatgcccagcttcaccatggcaaacaacctgcctatgcaacccccagtccccagtcagacctcctcatactcgtgcatgctgcccaccagcccgtcagtgaatgggcggagttatgatacctacacccctccgcacatgcaaacacacatgaacagtcagcccatgggcacctcggggaccacttcaacaggactcatttcacctggagtgtcagttcccgtccaagttcccgggagtgaacctgacatgtctcagtactggcctcgattacagtaa

SEQ ID NO: 37 - protein, 289 aa, Artificial Sequence
  Artificial Sequence
MMSYLKQPPYAVNGLSLTTSGMDLLHPSVGYPATPRKQRRERTTFTRAQLDVLEALFAKTRYPDIFMREEVALKINLPESRVQVWFKNRRAKCRQQQQQQQNGGQNKVRPAKKKTSPAREVSSESGTSGQFTPPSSTSVPTIASSSAPVSIWSPASISPLSDPLSTSSSCMQRSYPMTYTQASGYSQGYAGSTSYFGGMDCGSYLTPMHHQLPGPGATLSPMGTNAVTSHLNQSPASLSTQGYGASSLGFNSTTDCLDYKDQTASWKLNFNADCLDYKDQTSSWKFQVL

SEQ ID NO: 38 - protein, 297 aa, Artificial Sequence
  Artificial Sequence
MMSYLKQPPYAVNGLSLTTSGMDLLHPSVGYPGPWASCPAATPRKQRRERTTFTRAQLDVLEALFAKTRYPDIFMREEVALKINLPESRVQVWFKNRRAKCRQQQQQQQNGGQNKVRPAKKKSSPAREVSSESGTSGQFSPPSSTSVPTIASSSAPVSIWSPASISPLSDPLSTSSSCMQRSYPMTYTQASGYSQGYAGSTSYFGGMDCGSYLTPMHHQLPGPGATLSPMGTNAVTSHLNQSPASLSTQGYGASSLGFNSTTDCLDYKDQTASWKLNFNADCLDYKDQTSSWKFQVL

SEQ ID NO: 39 - DNA, 870 bp, Artificial Sequence
  Artificial Sequence
atgatgtcttatcttaagcaaccgccttacgcagtcaatgggctgagtctgaccacttcgggtatggacttgctgcacccctccgtgggctacccggccaccccccggaaacagcgccgggagaggacgacgttcactcgggcgcagctagatgtgctggaagcactgtttgccaagacccggtacccagacatcttcatgcgagaggaggtggcactgaaaatcaacttgcccgagtcgagggtgcaggtatggtttaagaatcgaagagctaagtgccgccaacaacagcaacaacagcagaatggaggtcaaaacaaagtgagacctgccaaaaagaagacatctccagctcgggaagtgagttcagagagtggaacaagtggccaattcactcccccctctagcacctcagtcccgaccattgccagcagcagtgctcctgtgtctatctggagcccagcttccatctccccactgtcagatcccttgtccacctcctcttcctgcatgcagaggtcctatcccatgacctatactcaggcttcaggttatagtcaaggatatgctggctcaacttcctactttgggggcatggactgtggatcatatttgacccctatgcatcaccagcttcccggaccaggggccacactcagtcccatgggtaccaatgcagtcaccagccatctcaatcagtccccagcttctctttccacccagggatatggagcttcaagcttgggttttaactcaaccactgattgcttggattataaggaccaaactgcctcctggaagcttaacttcaatgctgactgcttggattataaagatcagacatcctcgtggaaattccaggttttgtga

SEQ ID NO: 40 - DNA, 894 bp, Artificial Sequence
  Artificial Sequence
atgatgtcttatctaaagcaaccgccttacgcagtcaatgggctgagtctgaccacttcgggtatggacttgctgcatccctccgtgggctaccccgggccctgggcttcttgtcctgcagccaccccccggaaacagcgaagggagaggacgacatttactagggcacagctcgacgttctggaagctctgtttgccaagacccggtacccagacatcttcatgagggaagaggtggcactgaaaatcaacttgccagaatccagggtgcaggtatggtttaagaatcgaagagctaagtgccgccaacagcagcagcagcagcagaatggaggtcagaacaaagtgaggcctgccaagaagaagagctctccagctcgggaagtgagttcagagagtggaacaagtggccagttcagtcccccctctagtacctcagtcccaaccattgccagcagcagtgctccagtgtctatctggagcccagcgtccatctccccactgtctgaccccttgtccacttcctcctcctgcatgcagaggtcctatcccatgacctatactcaggcttcaggttatagtcaaggctatgctggctcaacttcctactttgggggcatggactgtggatcttatttgacccctatgcatcaccagcttcctggaccaggggccacactcagtcccatgggtaccaatgctgttaccagccatctcaatcagtccccagcttctctttccacccagggatatggagcttcaagcttgggttttaactcaaccactgattgcttggattataaggaccaaactgcctcttggaagcttaacttcaatgctgactgcttggattataaagatcagacgtcctcatggaaattccaggttttgtga

SEQ ID NO: 41 - protein, 236 aa, Artificial Sequence
  Artificial Sequence
MESSAKMESGGAGQQPQPQPQQPFLPPAACFFATAAAAAAAAAAAAAQSAQQQQQQQQQQQQAPQLRPAADGQPSGGGHKSAPKQVKRQRSSAPELMRCKRRLNFSGFGYSLPQQQPAAVARRNERERNRVKLVNLGFATLREHVPNGAANKKMSKVETLRSAVEYIRALQQLLDEHDAVSAAFQAGVLAPTIAPNYSNDLNSMAGAPVSSYSSDEGSYDPLAPEEQELLDFTNWF

SEQ ID NO: 42 - DNA, 2209 bp, Artificial Sequence
  Artificial Sequence
taatcccacctccctctctgtgctgggactcacagagggagacctcaggaggcagtctgtccatcacatgtccaaatgcagagcataccctgggctgggcgcagtggcgcacaactgtaattccagcactttgggaggctgatgtggaaggatcacttgagcccagaagttctagaccagcctgggcaacatggcaagaccctatctctacaaaaaaagttaaaaaatcagccacgtgtggtgacacacacctgtagtcccagctattcaggaggctgaggtgaggggatcacttaaggctgggaggttgaggctgcagtgagtcgtggttgcgccactgcactccagcctgggcaacagtgagaccctgtctcaaaagacaaaaaaaaaaaaaaaaaaaaaagaacatatcctggtgtggagtaggggacgctgctctgacagaggctcgggggcctgagctggctctgtgagctggggaggaggcagacagccaggccttgtctgcaagcagacctggcagcattgggctggccgccccccagggcctcctcttcatgcccagtgaatgactcaccttggcacagacacaatgttcggggtgggcacagtgcctgcttcccgccgcaccccagcccccctcaaatgccttccgagaagcccattgagcagggggcttgcattgcaccccagcctgacagcctggcatcttgggataaaagcagcacagccccctaggggctgcccttgctgtgtggcgccaccggcggtggagaacaaggctctattcagcctgtgcccaggaaaggggatcaggggatgcccaggcatggacagtgggtggcagggggggagaggagggctgtctgcttcccagaagtccaaggacacaaatgggtgaggggactgggcagggttctgaccctgtgggaccagagtggagggcgtagatggacctgaagtctccagggacaacagggcccaggtctcaggctcctagttgggcccagtggctccagcgtttccaaacccatccatccccagaggttcttcccatctctccaggctgatgtgtgggaactcgaggaaataaatctccagtgggagacggaggggtggccagggaaacggggcgctgcaggaataaagacgagccagcacagccagctcatgtgtaacggctttgtggagctgtcaaggcctggtctctgggagagaggcacagggaggccagacaaggaaggggtgacctggagggacagatccaggggctaaagtcctgataaggcaagagagtgccggccccctcttgccctatcaggacctccactgccacatagaggccatgattgacccttagacaaagggctggtgtccaatcccagcccccagccccagaactccagggaatgaatgggcagagagcaggaatgtgggacatctgtgttcaagggaaggactccaggagtctgctgggaatgaggcctagtaggaaatgaggtggcccttgagggtacagaacaggttcattcttcgccaaattcccagcaccttgcaggcacttacagctgagtgagataatgcctgggttatgaaatcaaaaagttggaaagcaggtcagaggtcatctggtacagcccttccttcccttttttttttttttttttgtgagacaaggtctctctctgttgcccaggctggagtggcgcaaacacagctcactgcagcctcaacctactgggctcaagcaatcctccagcctcagcctcccaaagtgctgggattacaagcatgagccaccccactcagccctttccttcctttttaattgatgcataataattgtaagtattcatcatggtccaaccaaccctttcttgacccaccttcctagagagagggtcctcttgcttcagcggtcagggccccagacccatggtctggctccaggtaccacctgcctcatgcaggagttggcgtgcccaggaagctctgcctctgggcacagtgacctcagtggggtgaggggagctctccccatagctgggctgcggcccaaccccaccccctcaggctatgccagggggtgttgccaggggcacccgggcatcgccagtctagcccactccttcataaagccctcgcatcccaggagcgagcagagccagagcaggttggagaggagacgcatcacctccgctgctcgcgg

SEQ ID NO: 43 - DNA, 683 bp, Artificial Sequence
  Artificial Sequence
aacatatcctggtgtggagtaggggacgctgctctgacagaggctcgggggcctgagctggctctgtgagctggggaggaggcagacagccaggccttgtctgcaagcagacctggcagcattgggctggccgccccccagggcctcctcttcatgcccagtgaatgactcaccttggcacagacacaatgttcggggtgggcacagtgcctgcttcccgccgcaccccagcccccctcaaatgccttccgagaagcccattgagcagggggcttgcattgcaccccagcctgacagcctggcatcttgggataaaagcagcacagccccctaggggctgcccttgctgtgtggcgccaccggcggtggagaacaaggctctattcagcctgtgcccaggaaaggggatcaggggatgcccaggcatggacagtgggtggcagggggggagaggagggctgtctgcttcccagaagtccaaggacacaaatgggtgaggggagagctctccccatagctgggctgcggcccaaccccaccccctcaggctatgccagggggtgttgccaggggcacccgggcatcgccagtctagcccactccttcataaagccctcgcatcccaggagcgagcagagccagagcaggttggagaggagacgcatcacctccgctgctcgcgg

SEQ ID NO: 44 - protein, 45 aa, Artificial Sequence
  Artificial Sequence
MLGDGDSPGPGFTPHDSAPYGALDMADFEFEQMFTDALGIDEYGG

SEQ ID NO: 45 - DNA, 135 bp, Artificial Sequence
  Artificial Sequence
atgttgggggacggggattccccgggtccgggatttaccccccacgactccgccccctacggcgctctggatatggccgacttcgagtttgagcagatgtttaccgatgcccttggaattgacgagtacggtggg

SEQ ID NO: 46 - DNA, 237 bp, Artificial Sequence
  Artificial Sequence
cgatggagcggagaatgggcggaactgggcggagttaggggcgggatgggcggagttaggggcgggactatggttgctgactaattgagatgcatgctttgcatacttctgcctgctggggagcctggggactttccacacctggttgctgactaattgagatgcatgctttgcatacttctgcctgctggggagcctggggactttccacaccctaactgacacacattccacagc